European Patent Application EP 4 417 702 A2, published August 21, 2024. Title: Method and System for predicting coupling probabilities of G-protein coupled receptors with G-proteins. Applicant: Cell Networks GmbH. The sequence listing filed with the application follows.

SEQUENCE LISTING (114 sequences)

SEQ ID NO: 1 - protein, 502 aa, Homo sapiens
MDYKDDDDKGSTLHNNSTTSPLFPNISSSWIHSPSDAGLPPGTVTHFGSYNVSRAAGNFSSPDGTTDDPLGGHTVWQVVFIAFLTGILALVTIIGNILVIVSFKVNKQLKTVNNYFLLSLACADLIIGVISMNLFTTYIIMNRWALGNLACDLWLAIDCVASNASVMNLLVISFDRYFSITRPLTYRAKRTTKRAGVMIGLAWVISFVLWAPAILFWQYFVGKRTVPPGECFIQFLSEPTITFGTAIAGFYMPVTIMTILYWRIYKETEKRTKELAGLQASGTEAETENFVHPTGSSRSCSSYELQQQSMKRSNRRKYGRCHFWFTTKSWKPSSEQMDQDHSSSDSWNNNDAAASLENSASSDEEDIGSETRAIYSIVLKLPGHSTILNSTKLPSSDNLQVPEEELGMVDLERKADKLQAQKSVDDGGSFPKSFSKLPIQLESAVDTAKTSDVNSSVGKSTATLPLSFKEATLAKRFALKTRSQITKRKRMSLVKEKKAAQT

SEQ ID NO: 2 - protein, 388 aa, Homo sapiens
MDYKDDDDKGSTLHNNSTTSPLFPNISSSWIHSPSDAGLPPGTVTHFGSYNVSRAAGNFSSPDGTTDDPLGGHTVWQVVFIAFLTGILALVTIIGNILVIVSFKVNKQLKTVNNYFLLSLACADLIIGVISMNLFTTYIIMNRWALGNLACDLWLAIDCVASNASVMNLLVISFDRYFSITRPLTYRAKRTTKRAGVMIGLAWVISFVLWAPAILFWQYFVGKRTVPPGECFIQFLSEPTITFGTAIAGFYMPVTIMTILYWRIYKETERTAKQNPLTEKSGVEKKAAQTLSAILLAFIITWTPYNIMVLVNTFCDSCIPKTFWNLGYWLCYINSTVNPVCYALCNKTFRTTFKMLLLCQCDKKKRRKQQYQQRQSVIFHKRAPEQAL

SEQ ID NO: 3 - protein, 383 aa, Homo sapiens
MDYKDDDDKGSTLHNNSTTSPLFPNISSSWIHSPSDAGLPPGTVTHFGSYNVSRAAGNFSSPDGTTDDPLGGHTVWQVVFIAFLTGILALVTIIGNILVIVSFKVNKQLKTVNNYFLLSLACADLIIGVISMNLFTTYIIMNRWALGNLACDLWLAIDCVASNASVMNLLVISFDRYFSITRPLTYRAKRTTKRAGVMIGLAWVISFVLWAPAILFWQYFVGKRTVPPGECFIQFLSEPTITFGTAIAGFYMPVTIMTILYWRIYKETEQSMGLSAAQEKKAAQTLSAILLAFIITWTPYNIMVLVNTFCDSCIPKTFWNLGYWLCYINSTVNPVCYALCNKTFRTTFKMLLLCQCDKKKRRKQQYQQRQSVIFHKRAPEQAL

SEQ ID NO: 4 - protein, 388 aa, Homo sapiens
MDYKDDDDKGSTLHNNSTTSPLFPNISSSWIHSPSDAGLPPGTVTHFGSYNVSRAAGNFSSPDGTTDDPLGGHTVWQVVFIAFLTGILALVTIIGNILVIVSVKVNKQLKTVNNYFLLSLACADLIIGVISMNLFTTYIIMNRWALGNLACDLWLAIDCVASNASVMNLLVISFDRYFSITRPLTYRAKRTTKRAGVMIGLAWVISFVLWAPAILFWQYFVGKRTVPPGECFIQFLSEPTITFGTAIAGFYMPVTIMTILYWRIYKETERTAKQNPLTEKSGVEKKAAQTLSAILLAFIITWTPYNIMVLVNTFCDSCIPKTFWNLGYWLCYINSTVNPVCYALCNKTFRTTFKMLLLCQCDKKKRRKQQYQQRQSVIFHKRAPEQAL

SEQ ID NO: 5 - protein, 582 aa, Homo sapiens
MGCLGNSKTEDQRNEEKAQREANKKIEKQLQKDKQVYRATHRLLLLGAGESGKSTIVKQMRILHVNGFNGEGGEEDPQAARSNSDGEKATKVQDIKNNLKEAIETIVAAMSNLGGSGGGGSGGSSSGGVFTLEDFVGDWEQTAAYNLDQVLEQGGVSSLLQNLAVSVTPIQRIVRSGENALKIDIHVIIPYEGLSADQMAQIEEVFKVVYPVDDHHFKVILPYGTLVIDGVTPNMLNYFGRPYEGIAVFDGKKITVTGTLWNGNKIIDERLITPDGSMLFRVTINSGGSGGGGSGGSSSGGVPPVELANPENQFRVDYILSVMNVPDFDFPPEFYEHAKALWEDEGVRACYERSNEYQLIDCAQYFLDKIDVIKQADYVPSDQDLLRCRVLTSGIFETKFQVDKVNFHMFDVGGQRDERRKWIQCFNDVTAIIFVVASSSYNMVIREDNQTNRLQEALNLFKSIWNNRWLRTISVILFLNKQDLLAEKVLAGKSKIEDYFPEFARYTTPEDATPEPGEDPRVTRAKYFIRDEFLRISTASGDGRHYCYPHFTCAVDTENIRRVFNDCRDIIQRMHLRQYELL

SEQ ID NO: 6 - protein, 542 aa, Homo sapiens
MGCTLSAEDKAAVERSKMIDRNLREDGEKAAREVKLLLLGAGESGKSTIVKQMKIIHEAGYSEEECKQYKAVVYSNTIQSIIAIIRAMGRLGGSGGGGSGGSSSGGVFTLEDFVGDWEQTAAYNLDQVLEQGGVSSLLQNLAVSVTPIQRIVRSGENALKIDIHVIIPYEGLSADQMAQIEEVFKVVYPVDDHHFKVILPYGTLVIDGVTPNMLNYFGRPYEGIAVFDGKKITVTGTLWNGNKIIDERLITPDGSMLFRVTINSGGSGGGGSGGSSSGGKIDFGDSARADDARQLFVLAGAAEEGFMTAELAGVIKRLWKDSGVQACFNRSREYQLNDSAAYYLNDLDRIAQPNYIPTQQDVLRTRVKTTGIVETHFTFKDLHFKMFDVGGQRSERKKWIHCFEGVTAIIFCVALSDYDLVLAEDEEMNRMHESMKLFDSICNNKWFTDTSIILFLNKKDLFEEKIKKSPLTICYPEYAGSNTYEEAAAYIQCQFEDLNKRKDTKEIYTHFTCATDTKNVQFVFDAVTDVIIKNNLKDCGLF

SEQ ID NO: 7 - protein, 543 aa, Homo sapiens
MGCTVSAEDKAAAERSKMIDKNLREDGEKAAREVKLLLLGAGESGKSTIVKQMKIIHEDGYSEEECRQYRAVVYSNTIQSIMAIVKAMGNLGGSGGGGSGGSSSGGVFTLEDFVGDWEQTAAYNLDQVLEQGGVSSLLQNLAVSVTPIQRIVRSGENALKIDIHVIIPYEGLSADQMAQIEEVFKVVYPVDDHHFKVILPYGTLVIDGVTPNMLNYFGRPYEGIAVFDGKKITVTGTLWNGNKIIDERLITPDGSMLFRVTINSGGSGGGGSGGSSSGGQIDFADPSRADDARQLFALSCTAEEQGVLPDDLSGVIRRLWADHGVQACFGRSREYQLNDSAAYYLNDLERIAQSDYIPTQQDVLRTRVKTTGIVETHFTFKDLHFKMFDVGGQRSERKKWIHCFEGVTAIIFCVALSAYDLVLAEDEEMNRMHESMKLFDSICNNKWFTDTSIILFLNKKDLFEEKITHSPLTICFPEYTGANKYDEAASYIQSKFEDLNKRKDTKEIYTHFTCATDTKNVQFVFDAVTDVIIKNNLKDCGLF

SEQ ID NO: 8 - protein, 542 aa, Homo sapiens
MGCTLSAEDKAAVERSKMIDRNLREDGEKAAKEVKLLLLGAGESGKSTIVKQMKIIHEDGYSEDECKQYKVVVYSNTIQSIIAIIRAMGRLGGSGGGGSGGSSSGGVFTLEDFVGDWEQTAAYNLDQVLEQGGVSSLLQNLAVSVTPIQRIVRSGENALKIDIHVIIPYEGLSADQMAQIEEVFKVVYPVDDHHFKVILPYGTLVIDGVTPNMLNYFGRPYEGIAVFDGKKITVTGTLWNGNKIIDERLITPDGSMLFRVTINSGGSGGGGSGGSSSGGKIDFGEAARADDARQLFVLAGSAEEGVMTPELAGVIKRLWRDGGVQACFSRSREYQLNDSASYYLNDLDRISQSNYIPTQQDVLRTRVKTTGIVETHFTFKDLYFKMFDVGGQRSERKKWIHCFEGVTAIIFCVALSDYDLVLAEDEEMNRMHESMKLFDSICNNKWFTETSIILFLNKKDLFEEKIKRSPLTICYPEYTGSNTYEEAAAYIQCQFEDLNRRKDTKEIYTHFTCATDTKNVQFVFDAVTDVIIKNNLKECGLY

SEQ ID NO: 9 - protein, 542 aa, Homo sapiens
MGCTLSAEERAALERSKAIEKNLKEDGISAAKDVKLLLLGAGESGKSTIVKQMKIIHEDGFSGEDVKQYKPVVYSNTIQSLAAIVRAMDTLGGSGGGGSGGSSSGGVFTLEDFVGDWEQTAAYNLDQVLEQGGVSSLLQNLAVSVTPIQRIVRSGENALKIDIHVIIPYEGLSADQMAQIEEVFKVVYPVDDHHFKVILPYGTLVIDGVTPNMLNYFGRPYEGIAVFDGKKITVTGTLWNGNKIIDERLITPDGSMLFRVTINSGGSGGGGSGGSSSGGGIEYGDKERKADAKMVCDVVSRMEDTEPFSAELLSAMMRLWGDSGIQECFNRSREYQLNDSAKYYLDSLDRIGAADYQPTEQDILRTRVKTTGIVETHFTFKNLHFRLFDVGGQRSERKKWIHCFEDVTAIIFCVALSGYDQVLHEDETTNRMHESLMLFDSICNNKFFIDTSIILFLNKKDLFGEKIKKSPLTICFPEYTGPNTYEDAAAYIQAQFESKNRSPNKEIYCHMTCATDTNNIQVVFDAVTDIIIANNLRGCGLY

SEQ ID NO: 10 - protein, 547 aa, Homo sapiens
MTLESIMACCLSEEAKEARRINDEIERQLRRDKRDARRELKLLLLGTGESGKSTFIKQMRIIHGSGYSDEDKRGFTKLVYQNIFTAMQAMIRAMDTLGGSGGGGSGGSSSGGVFTLEDFVGDWEQTAAYNLDQVLEQGGVSSLLQNLAVSVTPIQRIVRSGENALKIDIHVIIPYEGLSADQMAQIEEVFKVVYPVDDHHFKVILPYGTLVIDGVTPNMLNYFGRPYEGIAVFDGKKITVTGTLWNGNKIIDERLITPDGSMLFRVTINSGGSGGGGSGGSSSGGKIPYKYEHNKAHAQLVREVDVEKVSAFENPYVDAIKSLWNDPGIQECYDRRREYQLSDSTKYYLNDLDRVADPAYLPTQQDVLRVRVPTTGIIEYPFDLQSVIFRMVDVGGQRSERRKWIHCFENVTSIMFLVALSEYDQVLVESDNENRMEESKALFRTIITYPWFQNSSVILFLNKKDLLEEKIMYSHLVDYFPEYDGPQRDAQAAREFILKMFVDLNPDSDKIIYSHFTCATDTENIRFVFAAVKDTILQLNLKEYNLV

SEQ ID NO: 11 - protein, 547 aa, Homo sapiens
MTLESMMACCLSDEVKESKRINAEIEKQLRRDKRDARRELKLLLLGTGESGKSTFIKQMRIIHGAGYSEEDKRGFTKLVYQNIFTAMQAMIRAMETLGGSGGGGSGGSSSGGVFTLEDFVGDWEQTAAYNLDQVLEQGGVSSLLQNLAVSVTPIQRIVRSGENALKIDIHVIIPYEGLSADQMAQIEEVFKVVYPVDDHHFKVILPYGTLVIDGVTPNMLNYFGRPYEGIAVFDGKKITVTGTLWNGNKIIDERLITPDGSMLFRVTINSGGSGGGGSGGSSSGGKILYKYEQNKANALLIREVDVEKVTTFEHQYVSAIKTLWEDPGIQECYDRRREYQLSDSAKYYLTDVDRIATLGYLPTQQDVLRVRVPTTGIIEYPFDLENIIFRMVDVGGQRSERRKWIHCFENVTSIMFLVALSEYDQVLVESDNENRMEESKALFRTIITYPWFQNSSVILFLNKKDLLEDKILYSHLVDYFPEFDGPQRDAQAAREFILKMFVDLNPDSDKIIYSHFTCATDTENIRFVFAAVKDTILQLNLKEYNLV

SEQ ID NO: 12 - protein, 543 aa, Homo sapiens
MAGCCCLSAEEKESQRISAEIERQLRRDKKDARRELKLLLLGTGESGKSTFIKQMRIIHGSGYSDEDRKGFTKLVYQNIFTAMQAMIRAMDTLGGSGGGGSGGSSSGGVFTLEDFVGDWEQTAAYNLDQVLEQGGVSSLLQNLAVSVTPIQRIVRSGENALKIDIHVIIPYEGLSADQMAQIEEVFKVVYPVDDHHFKVILPYGTLVIDGVTPNMLNYFGRPYEGIAVFDGKKITVTGTLWNGNKIIDERLITPDGSMLFRVTINSGGSGGGGSGGSSSGGRIQYVCEQNKENAQIIREVEVDKVSMLSREQVEAIKQLWQDPGIQECYDRRREYQLSDSAKYYLTDIDRIATPSFVPTQQDVLRVRVPTTGIIEYPFDLENIIFRMVDVGGQRSERRKWIHCFESVTSIIFLVALSEYDQVLAECDNENRMEESKALFKTIITYPWFLNSSVILFLNKKDLLEEKIMYSHLISYFPEYTGPKQDVRAARDFILKLYQDQNPDKEKVIYSHFTCATDTDNIRFVFAAVKDTILQLNLREFNLV

SEQ ID NO: 13 - protein, 562 aa, Homo sapiens
MARSLTWRCCPWCLTEDEKAAARVDQEINRILLEQKKQDRGELKLLLLGPGESGKSTFIKQMRIIHGAGYSEEERKGFRPLVYQNIFVSMRAMIEAMERLGGSGGGGSGGSSSGGVFTLEDFVGDWEQTAAYNLDQVLEQGGVSSLLQNLAVSVTPIQRIVRSGENALKIDIHVIIPYEGLSADQMAQIEEVFKVVYPVDDHHFKVILPYGTLVIDGVTPNMLNYFGRPYEGIAVFDGKKITVTGTLWNGNKIIDERLITPDGSMLFRVTINSGGSGGGGSGGSSSGGQIPFSRPESKHHASLVMSQDPYKVTTFEKRYAAAMQWLWRDAGIRAYYERRREFHLLDSAVYYLSHLERITEEGYVPTAQDVLRSRMPTTGINEYCFSVQKTNLRIVDVGGQKSERKKWIHCFENVIALIYLASLSEYDQCLEENNQENRMKESLALFGTILELPWFKSTSVILFLNKTDILEEKIPTSHLATYFPSFQGPKQDAEAAKRFILDMYTRMYTGCVDGPEGSKKGARSRRLFSHYTCATDTQNIRKVFKDVRDSVLARYLDEINLL

SEQ ID NO: 14 - protein, 569 aa, Homo sapiens
MSGVVRTLSRCLLPAEAGGARERRAGSGARDAEREARRRSRDIDALLARERRAVRRLVKILLLGAGESGKSTFLKQMRIIHGREFDQKALLEFRDTIFDNILKGSRVLVDARDKLGGSGGGGSGGSSSGGVFTLEDFVGDWEQTAAYNLDQVLEQGGVSSLLQNLAVSVTPIQRIVRSGENALKIDIHVIIPYEGLSADQMAQIEEVFKVVYPVDDHHFKVILPYGTLVIDGVTPNMLNYFGRPYEGIAVFDGKKITVTGTLWNGNKIIDERLITPDGSMLFRVTINSGGSGGGGSGGSSSGGGIPWQYSENEKHGMFLMAFENKAGLPVEPATFQLYVPALSALWRDSGIREAFSRRSEFQLGESVKYFLDNLDRIGQLNYFPSKQDILLARKATKGIVEHDFVIKKIPFKMVDVGGQRSQRQKWFQCFDGITSILFMVSSSEYDQVLMEDRRTNRLVESMNIFETIVNNKLFFNVSIILFLNKMDLLVEKVKTVSIKKHFPDFRGDPHRLEDVQRYLVQCFDRKRRNRSKPLFHHFTTAIDTENVRFVFHAVKDTILQENLKDIMLQ

SEQ ID NO: 15 - protein, 565 aa, Homo sapiens
MADFLPSRSVLSVCFPGCLLTSGEAEQQRKSKEIDKCLSREKTYVKRLVKILLLGAGESGKSTFLKQMRIIHGQDFDQRAREEFRPTIYSNVIKGMRVLVDAREKLGGSGGGGSGGSSSGGVFTLEDFVGDWEQTAAYNLDQVLEQGGVSSLLQNLAVSVTPIQRIVRSGENALKIDIHVIIPYEGLSADQMAQIEEVFKVVYPVDDHHFKVILPYGTLVIDGVTPNMLNYFGRPYEGIAVFDGKKITVTGTLWNGNKIIDERLITPDGSMLFRVTINSGGSGGGGSGGSSSGGHIPWGDNSNQQHGDKMMSFDTRAPMAAQGMVETRVFLQYLPAIRALWADSGIQNAYDRRREFQLGESVKYFLDNLDKLGEPDYIPSQQDILLARRPTKGIHEYDFEIKNVPFKMVDVGGQRSERKRWFECFDSVTSILFLVSSSEFDQVLMEDRLTNRLTESLNIFETIVNNRVFSNVSIILFLNKTDLLEEKVQIVSIKDYFLEFEGDPHCLRDVQKFLVECFRNKRRDQQQKPLYHHFTTAINTENIRLVFRDVKDTILHDNLKQLMLQ

SEQ ID NO: 16 - protein, 366 aa, Homo sapiens
MVTGYRLFEEILGGSGGGGSGGSSSGGSELDQLRQEAEQLKNQIRDARKACADATLSQITNNIDPVGRIQMRTRRTLRGHLAKIYAMHWGTDSRLLVSASQDGKLIIWDSYTTNKVHAIPLRSSWVMTCAYAPSGNYVACGGLDNICSIYNLKTREGNVRVSRELAGHTGYLSCCRFLDDNQIVTSSGDTTCALWDIETGQQTTTFTGHTGDVMSLSLAPDTRLFVSGACDASAKLWDVREGMCRQTFTGHESDINAICFFPNGNAFATGSDDATCRLFDLRADQELMTYSHDNIICGITSVSFSKSGRLLLAGYDDFNCNVWDALKADRAGVLAGHDNRVSCLGVTDDGMAVATGSWDSFLKIWN

SEQ ID NO: 17 - protein, 366 aa, Homo sapiens
MVTGYRLFEEILGGSGGGGSGGSSSGGSELEQLRQEAEQLRNQIRDARKACGDSTLTQITAGLDPVGRIQMRTRRTLRGHLAKIYAMHWGTDSRLLVSASQDGKLIIWDSYTTNKVHAIPLRSSWVMTCAYAPSGNFVACGGLDNICSIYSLKTREGNVRVSRELPGHTGYLSCCRFLDDNQIITSSGDTTCALWDIETGQQTVGFAGHSGDVMSLSLAPDGRTFVSGACDASIKLWDVRDSMCRQTFIGHESDINAVAFFPNGYAFTTGSDDATCRLFDLRADQELLMYSHDNIICGITSVAFSRSGRLLLAGYDDFNCNIWDAMKGDRAGVLAGHDNRVSCLGVTDDGMAVATGSWDSFLKIWN

SEQ ID NO: 18 - protein, 366 aa, Homo sapiens
MVTGYRLFEEILGGSGGGGSGGSSSGGGEMEQLRQEAEQLKKQIADARKACADVTLAELVSGLEVVGRVQMRTRRTLRGHLAKIYAMHWATDSKLLVSASQDGKLIVWDSYTTNKVHAIPLRSSWVMTCAYAPSGNFVACGGLDNMCSIYNLKSREGNVKVSRELSAHTGYLSCCRFLDDNNIVTSSGDTTCALWDIETGQQKTVFVGHTGDCMSLAVSPDFNLFISGACDASAKLWDVREGTCRQTFTGHESDINAICFFPNGEAICTGSDDASCRLFDLRADQELICFSHESIICGITSVAFSLSGRLLFAGYDDFNCNVWDSMKSERVGILSGHDNRVSCLGVTADGMAVATGSWDSFLKIWN

SEQ ID NO: 19 - protein, 366 aa, Homo sapiens
MVTGYRLFEEILGGSGGGGSGGSSSGGSELEQLRQEAEQLRNQIQDARKACNDATLVQITSNMDSVGRIQMRTRRTLRGHLAKIYAMHWGYDSRLLVSASQDGKLIIWDSYTTNKMHAIPLRSSWVMTCAYAPSGNYVACGGLDNICSIYNLKTREGNVRVSRELPGHTGYLSCCRFLDDSQIVTSSGDTTCALWDIETAQQTTTFTGHSGDVMSLSLSPDMRTFVSGACDASSKLWDIRDGMCRQSFTGHVSDINAVSFFPNGYAFATGSDDATCRLFDLRADQELLLYSHDNIICGITSVAFSKSGRLLLAGYDDFNCNVWDTLKGDRAGVLAGHDNRVSCLGVTDDGMAVATGSWDSFLRIWN

SEQ ID NO: 20 - protein, 421 aa, Homo sapiens
MVTGYRLFEEILGGSGGGGSGGSSSGGCDQTFLVNVFGSCDKCFKQRALRPVFKKSQQLSYCSTCAEIMATEGLHENETLASLKSEAESLKGKLEEERAKLHDVELHQVAERVEALGQFVMKTRRTLKGHGNKVLCMDWCKDKRRIVSSSQDGKVIVWDSFTTNKEHAVTMPCTWVMACAYAPSGCAIACGGLDNKCSVYPLTFDKNENMAAKKKSVAMHTNYLSACSFTNSDMQILTASGDGTCALWDVESGQLLQSFHGHGADVLCLDLAPSETGNTFVSGGCDKKAMVWDMRSGQCVQAFETHESDINSVRYYPSGDAFASGSDDATCRLYDLRADREVAIYSKESIIFGASSVDFSLSGRLLFAGYNDYTINVWDVLKGSRVSILFGHENRVSTLRVSPDGTAFCSGSWDHTLRVWA

SEQ ID NO: 21 - protein, 97 aa, Homo sapiens
MVTGYRLFEEILGGSGGGGSGGSSSGGASNNTASIAQARKLVEQLKMEANIDRIKVSKAAADLMAYCEAHAKEDPLLTPVPASENPFREKKFFCAIL

SEQ ID NO: 22 - protein, 101 aa, Homo sapiens
MVTGYRLFEEILGGSGGGGSGGSSSGGKGETPVNSTMSIGQARKMVEQLKIEASLCRIKVSKAAADLMTYCDAHACEDPLITPVPTSENPFREKKFFCALL

SEQ ID NO: 23 - protein, 101 aa, Homo sapiens
MVTGYRLFEEILGGSGGGGSGGSSSGGKEGMSNNSTTSISQARKAVEQLKMEACMDRVKVSQAAADLLAYCEAHVREDPLIIPVPASENPFREKKFFCTIL

SEQ ID NO: 24 - protein, 94 aa, Homo sapiens
MVTGYRLFEEILGGSGGGGSGGSSSGGSGSSSVAAMKKVVQQLRLEAGLNRVKVSQAAADLKQFCLQNAQHDPLLTGVSSSTNPFRPQKVCSFL

SEQ ID NO: 25 - protein, 94 aa, Homo sapiens
MVTGYRLFEEILGGSGGGGSGGSSSGGSATNNIAQARKLVEQLRIEAGIERIKVSKAASDLMSYCEQHARNDPLLVGVPASENPFKDKKPCIIL

SEQ ID NO: 26 - protein, 96 aa, Homo sapiens
MVTGYRLFEEILGGSGGGGSGGSSSGGSNNMAKIAEARKTVEQLKLEVNIDRMKVSQAAAELLAFCETHAKDDPLVTPVPAAENPFRDKRLFCVLL

SEQ ID NO: 27 - protein, 94 aa, Homo sapiens
MVTGYRLFEEILGGSGGGGSGGSSSGGSSGASASALQRLVEQLKLEAGVERIKVSQAAAELQQYCMQNACKDALLVGVPAGSNPFREPRSCALL

SEQ ID NO: 28 - protein, 99 aa, Homo sapiens
MVTGYRLFEEILGGSGGGGSGGSSSGGPALHIEDLPEKEKLKMEVEQLRKEVKLQRQQVSKCSEEIKNYIEERSGEDPLVKGIPEDKNPFKEKGSCVIS

SEQ ID NO: 29 - protein, 98 aa, Homo sapiens
MVTGYRLFEEILGGSGGGGSGGSSSGGSSKTASTNNIAQARRTVQQLRLEASIERIKVSKASADLMSYCEEHARSDPLLIGIPTSENPFKDKKTCIIL

SEQ ID NO: 30 - protein, 93 aa, Homo sapiens
MVTGYRLFEEILGGSGGGGSGGSSSGGEEWDVPQMKKEVESLKYQLAFQREMASKTIPELLKWIEDGIPKDPFLNPDLMKNNPWVEKGKCTIL

SEQ ID NO: 31 - protein, 100 aa, Homo sapiens
MVTGYRLFEEILGGSGGGGSGGSSSGGPVINIEDLTEKDKLKMEVDQLKKEVTLERMLVSKCCEEVRDYVEERSGEDPLVKGIPEDKNPFKELKGGCVIS

SEQ ID NO: 32 - protein, 95 aa, Homo sapiens
MVTGYRLFEEILGGSGGGGSGGSSSGGAQDLSEKDLLKMEVEQLKKEVKNTRIPISKAGKEIKEYVEAQAGNDPFLKGIPEDKNPFKEKGGCLIS

SEQ ID NO: 33 - protein, 435 aa, Homo sapiens
MGCLGNSKTEDQRNEEKAQREANKKIEKQLQKDKQVYRATHRLLLLGAGESGKSTIVKQMRILHVNGFNGEGGEEDPQAARSNSDGEKATKVQDIKNNLKEAIETIVAAMSNLGGSGGGGSGGSSSGGVTGYRLFEEILGGSGGGGSGGSSSGGVPPVELANPENQFRVDYILSVMNVPDFDFPPEFYEHAKALWEDEGVRACYERSNEYQLIDCAQYFLDKIDVIKQADYVPSDQDLLRCRVLTSGIFETKFQVDKVNFHMFDVGGQRDERRKWIQCFNDVTAIIFVVASSSYNMVIREDNQTNRLQEALNLFKSIWNNRWLRTISVILFLNKQDLLAEKVLAGKSKIEDYFPEFARYTTPEDATPEPGEDPRVTRAKYFIRDEFLRISTASGDGRHYCYPHFTCAVDTENIRRVFNDCRDIIQRMHLRQYELL

SEQ ID NO: 34 - protein, 568 aa, Homo sapiens
MGCLGNSKTEDQRNEEKAQREANKKIEKQLQKDKQVYRATHRLLLLGAGESGKSTIVKQMRILHVNGFNGDSEKATKVQDIKNNLKEAIETIVAAMSNLVPPVELANPENQFRVDYILSVMNVPDFGGSGGGGSGGSSSGGVFTLEDFVGDWEQTAAYNLDQVLEQGGVSSLLQNLAVSVTPIQRIVRSGENALKIDIHVIIPYEGLSADQMAQIEEVFKVVYPVDDHHFKVILPYGTLVIDGVTPNMLNYFGRPYEGIAVFDGKKITVTGTLWNGNKIIDERLITPDGSMLFRVTINSGGSGGGGSGGSSSGGDFPPEFYEHAKALWEDEGVRACYERSNEYQLIDCAQYFLDKIDVIKQADYVPSDQDLLRCRVLTSGIFETKFQVDKVNFHMFDVGGQRDERRKWIQCFNDVTAIIFVVASSSYNMVIREDNQTNRLQEALNLFKSIWNNRWLRTISVILFLNKQDLLAEKVLAGKSKIEDYFPEFARYTTPEDATPEPGEDPRVTRAKYFIRDEFLRISTASGDGRHYCYPHFTCAVDTENIRRVFNDCRDIIQRMHLRQYELL

SEQ ID NO: 35 - protein, 421 aa, Homo sapiens
MGCLGNSKTEDQRNEEKAQREANKKIEKQLQKDKQVYRATHRLLLLGAGESGKSTIVKQMRILHVNGFNGDSEKATKVQDIKNNLKEAIETIVAAMSNLVPPVELANPENQFRVDYILSVMNVPDFGGSGGGGSGGSSSGGVTGYRLFEEILGGSGGGGSGGSSSGGDFPPEFYEHAKALWEDEGVRACYERSNEYQLIDCAQYFLDKIDVIKQADYVPSDQDLLRCRVLTSGIFETKFQVDKVNFHMFDVGGQRDERRKWIQCFNDVTAIIFVVASSSYNMVIREDNQTNRLQEALNLFKSIWNNRWLRTISVILFLNKQDLLAEKVLAGKSKIEDYFPEFARYTTPEDATPEPGEDPRVTRAKYFIRDEFLRISTASGDGRHYCYPHFTCAVDTENIRRVFNDCRDIIQRMHLRQYELL

SEQ ID NO: 36 - protein, 582 aa, Homo sapiens
MASLGNSKTEDQRNEEKAQREANKKIEKQLQKDKQVYRATHRLLLLGAGESGKSTIVKQMRILHVNGFNGEGGEEDPQAARSNSDGEKATKVQDIKNNLKEAIETIVAAMSNLGGSGGGGSGGSSSGGVFTLEDFVGDWEQTAAYNLDQVLEQGGVSSLLQNLAVSVTPIQRIVRSGENALKIDIHVIIPYEGLSADQMAQIEEVFKVVYPVDDHHFKVILPYGTLVIDGVTPNMLNYFGRPYEGIAVFDGKKITVTGTLWNGNKIIDERLITPDGSMLFRVTINSGGSGGGGSGGSSSGGVPPVELANPENQFRVDYILSVMNVPDFDFPPEFYEHAKALWEDEGVRACYERSNEYQLIDCAQYFLDKIDVIKQADYVPSDQDLLRCRVLTSGIFETKFQVDKVNFHMFDVGGQRDERRKWIQCFNDVTAIIFVVASSSYNMVIREDNQTNRLQEALNLFKSIWNNRWLRTISVILFLNKQDLLAEKVLAGKSKIEDYFPEFARYTTPEDATPEPGEDPRVTRAKYFIRDEFLRISTASGDGRHYCYPHFTCAVDTENIRRVFNDCRDIIQRMHLRQYELL

SEQ ID NO: 37 - protein, 547 aa, Homo sapiens
MTLESIMACCLSEEAKEARRINDEIERQLRRDKRDARRELKLLLLGTGESGKSTFIKQMRIIHGSGYSDEDKRGFTKLVYQNIFTAMQAMIRAMDTLGGSGGGGSGGSSSGGVFTLEDFVGDWEQTAAYNLDQVLEQGGVSSLLQNLAVSVTPIQRIVRSGENALKIDIHVIIPYEGLSADQMAQIEEVFKVVYPVDDHHFKVILPYGTLVIDGVTPNMLNYFGRPYEGIAVFDGKKITVTGTLWNGNKIIDERLITPDGSMLFRVTINSGGSGGGGSGGSSSGGKIPYKYEHNKAHAQLVREVDVEKVSAFENPYVDAIKSLWNDPGIQECYDRRREYQLSDSTKYYLNDLDRVADPAYLPTQQDVLRVCVPTTGIIEYPFDLQSVIFRMVDVGGQRSERRKWIHCFENVTSIMFLVALSEYDQVLVESDNENRMEESKALFRTIITYPWFQNSSVILFLNKKDLLEEKIMYSHLVDYFPEYDGPQRDAQAAREFILKMFVDLNPDSDKIIYSHFTCATDTENIRFVFAAVKDTILQLNLKEYNLV

SEQ ID NO: 38 - protein, 547 aa, Homo sapiens
MTLESIMACCLSEEAKEARRINDEIERQLRRDKRDARRELKLLLLGTGESGKSTFIKQMRIIHGSGYSDEDKRGFTKLVYQNIFTAMQAMIRAMDTLKIPYKYEHNKAHAQLVREVDVEKVSAGGSGGGGSGGSSSGGVFTLEDFVGDWEQTAAYNLDQVLEQGGVSSLLQNLAVSVTPIQRIVRSGENALKIDIHVIIPYEGLSADQMAQIEEVFKVVYPVDDHHFKVILPYGTLVIDGVTPNMLNYFGRPYEGIAVFDGKKITVTGTLWNGNKIIDERLITPDGSMLFRVTINSGGSGGGGSGGSSSGGFENPYVDAIKSLWNDPGIQECYDRRREYQLSDSTKYYLNDLDRVADPAYLPTQQDVLRVRVPTTGIIEYPFDLQSVIFRMVDVGGQRSERRKWIHCFENVTSIMFLVALSEYDQVLVESDNENRMEESKALFRTIITYPWFQNSSVILFLNKKDLLEEKIMYSHLVDYFPEYDGPQRDAQAAREFILKMFVDLNPDSDKIIYSHFTCATDTENIRFVFAAVKDTILQLNLKEYNLV

SEQ ID NO: 39 - protein, 547 aa, Homo sapiens
MTLESMMACCLSDEVKESKRINAEIEKQLRRDKRDARRELKLLLLGTGESGKSTFIKQMRIIHGAGYSEEDKRGFTKLVYQNIFTAMQAMIRAMETLKILYKYEQNKANALLIREVDVEKVTTGGSGGGGSGGSSSGGVFTLEDFVGDWEQTAAYNLDQVLEQGGVSSLLQNLAVSVTPIQRIVRSGENALKIDIHVIIPYEGLSADQMAQIEEVFKVVYPVDDHHFKVILPYGTLVIDGVTPNMLNYFGRPYEGIAVFDGKKITVTGTLWNGNKIIDERLITPDGSMLFRVTINSGGSGGGGSGGSSSGGFEHQYVSAIKTLWEDPGIQECYDRRREYQLSDSAKYYLTDVDRIATLGYLPTQQDVLRVRVPTTGIIEYPFDLENIIFRMVDVGGQRSERRKWIHCFENVTSIMFLVALSEYDQVLVESDNENRMEESKALFRTIITYPWFQNSSVILFLNKKDLLEDKILYSHLVDYFPEFDGPQRDAQAAREFILKMFVDLNPDSDKIIYSHFTCATDTENIRFVFAAVKDTILQLNLKEYNLV

SEQ ID NO: 40 - protein, 543 aa, Homo sapiens
MAGCCCLSAEEKESQRISAEIERQLRRDKKDARRELKLLLLGTGESGKSTFIKQMRIIHGSGYSDEDRKGFTKLVYQNIFTAMQAMIRAMDTLRIQYVCEQNKENAQIIREVEVDKVSMGGSGGGGSGGSSSGGVFTLEDFVGDWEQTAAYNLDQVLEQGGVSSLLQNLAVSVTPIQRIVRSGENALKIDIHVIIPYEGLSADQMAQIEEVFKVVYPVDDHHFKVILPYGTLVIDGVTPNMLNYFGRPYEGIAVFDGKKITVTGTLWNGNKIIDERLITPDGSMLFRVTINSGGSGGGGSGGSSSGGLSREQVEAIKQLWQDPGIQECYDRRREYQLSDSAKYYLTDIDRIATPSFVPTQQDVLRVRVPTTGIIEYPFDLENIIFRMVDVGGQRSERRKWIHCFESVTSIIFLVALSEYDQVLAECDNENRMEESKALFKTIITYPWFLNSSVILFLNKKDLLEEKIMYSHLISYFPEYTGPKQDVRAARDFILKLYQDQNPDKEKVIYSHFTCATDTDNIRFVFAAVKDTILQLNLREFNLV

SEQ ID NO: 41 - protein, 562 aa, Homo sapiens
MARSLTWRCCPWCLTEDEKAAARVDQEINRILLEQKKQDRGELKLLLLGPGESGKSTFIKQMRIIHGAGYSEEERKGFRPLVYQNIFVSMRAMIEAMERLQIPFSRPESKHHASLVMSQDPYKVTTGGSGGGGSGGSSSGGVFTLEDFVGDWEQTAAYNLDQVLEQGGVSSLLQNLAVSVTPIQRIVRSGENALKIDIHVIIPYEGLSADQMAQIEEVFKVVYPVDDHHFKVILPYGTLVIDGVTPNMLNYFGRPYEGIAVFDGKKITVTGTLWNGNKIIDERLITPDGSMLFRVTINSGGSGGGGSGGSSSGGFEKRYAAAMQWLWRDAGIRAYYERRREFHLLDSAVYYLSHLERITEEGYVPTAQDVLRSRMPTTGINEYCFSVQKTNLRIVDVGGQKSERKKWIHCFENVIALIYLASLSEYDQCLEENNQENRMKESLALFGTILELPWFKSTSVILFLNKTDILEEKIPTSHLATYFPSFQGPKQDAEAAKRFILDMYTRMYTGCVDGPEGSKKGARSRRLFSHYTCATDTQNIRKVFKDVRDSVLARYLDEINLL

SEQ ID NO: 42 - protein, 513 aa, Homo sapiens
MVFTLEDFVGDWEQTAAYNLDQVLEQGGVSSLLQNLAVSVTPIQRIVRSGENALKIDIHVIIPYEGLSADQMAQIEEVFKVVYPVDDHHFKVILPYGTLVIDGVTPNMLNYFGRPYEGIAVFDGKKITVTGTLWNGNKIIDERLITPDGSMLFRVTINSGGSGGGGSGGSSSGGSELDQLRQEAEQLKNQIRDARKACADATLSQITNNIDPVGRIQMRTRRTLRGHLAKIYAMHWGTDSRLLVSASQDGKLIIWDSYTTNKVHAIPLRSSWVMTCAYAPSGNYVACGGLDNICSIYNLKTREGNVRVSRELAGHTGYLSCCRFLDDNQIVTSSGDTTCALWDIETGQQTTTFTGHTGDVMSLSLAPDTRLFVSGACDASAKLWDVREGMCRQTFTGHESDINAICFFPNGNAFATGSDDATCRLFDLRADQELMTYSHDNIICGITSVSFSKSGRLLLAGYDDFNCNVWDALKADRAGVLAGHDNRVSCLGVTDDGMAVATGSWDSFLKIWN

SEQ ID NO: 43 - protein, 244 aa, Homo sapiens
MVFTLEDFVGDWEQTAAYNLDQVLEQGGVSSLLQNLAVSVTPIQRIVRSGENALKIDIHVIIPYEGLSADQMAQIEEVFKVVYPVDDHHFKVILPYGTLVIDGVTPNMLNYFGRPYEGIAVFDGKKITVTGTLWNGNKIIDERLITPDGSMLFRVTINSGGSGGGGSGGSSSGGASNNTASIAQARKLVEQLKMEANIDRIKVSKAAADLMAYCEAHAKEDPLLTPVPASENPFREKKFFCAIL

SEQ ID NO: 44 - protein, 97 aa, Homo sapiens
MVTGYRLFEEILGGSGGGGSGGSSSGGASNNTASIAQARKLVEQLKMEANIDRIKVSKAAADLMAYCEAHAKEDPLLTPVPASENPFREKKFFSAIL

SEQ ID NO: 45 - protein, 1242 aa, Homo sapiens
MVTGYRLFEEILGGSGGGGSGGSSSGGAGAQPGVHALQLKPVCVSDSLKKGTKFVKWDDDSTIVTPIILRTDPQGFFFYWTDQNKETELLDLSLVKDARCGRHAKAPKDPKLRELLDVGNIGRLEQRMITVVYGPDLVNISHLNLVAFQEEVAKEWTNEVFSLATNLLAQNMSRDAFLEKAYTKLKLQVTPEGRIPLKNIYRLFSADRKRVETALEACSLPSSRNDSIPQEDFTPEVYRVFLNNLCPRPEIDNIFSEFGAKSKPYLTVDQMMDFINLKQRDPRLNEILYPPLKQEQVQVLIEKYEPNNSLARKGQISVDGFMRYLSGEENGVVSPEKLDLNEDMSQPLSHYFINSSHNTYLTAGQLAGNSSVEMYRQVLLSGCRCVELDCWKGRTAEEEPVITHGFTMTTEISFKEVIEAIAECAFKTSPFPILLSFENHVDSPKQQAKMAEYCRLIFGDALLMEPLEKYPLESGVPLPSPMDLMYKILVKNKKKSHKSSEGSGKKKLSEQASNTYSDSSSMFEPSSPGAGEADTESDDDDDDDDCKKSSMDEGTAGSEAMATEEMSNLVNYIQPVKFESFEISKKRNKSFEMSSFVETKGLEQLTKSPVEFVEYNKMQLSRIYPKGTRVDSSNYMPQLFWNAGCQMVALNFQTMDLAMQINMGMYEYNGKSGYRLKPEFMRRPDKHFDPFTEGIVDGIVANTLSVKIISGQFLSDKKVGTYVEVDMFGLPVDTRRKAFKTKTSQGNAVNPVWEEEPIVFKKVVLPTLACLRIAVYEEGGKFIGHRILPVQAIRPGYHYICLRNERNQPLTLPAVFVYIEVKDYVPDTYADVIEALSNPIRYVNLMEQRAKQLAALTLEDEEEVKKEADPGETPSEAPSEARTTPAENGVNHTTTLTPKPPSQALHSQPAPGSVKAPAKTEDLIQSVLTEVEAQTIEELKQQKSFVKLQKKHYKEMKDLVKRHHKKTTDLIKEHTTKYNEIQNDYLRRRAALEKSAKKDSKKKSEPSSPDHGSSTIEQDLAALDAEMTQKLIDLKDKQQQQLLNLRQEQYYSEKYQKREHIKLLIQKLTDVAEECQNNQLKKLKEICEKEKKELKKKMDKKRQEKITEAKSKDKSQMEEEKTEMIRSYIQEVVQYIKRLEEAQSKRQEKLVEKHKEIRQQILDEKPKLQVELEQEYQDKFKRLPLEILEFVQEAMKGKISEDSNHGSAPLSLSSDPGKVNHKTPSSEELGGDIPGKEFDTPL

SEQ ID NO: 46 - protein, 1207 aa, Homo sapiens
MVTGYRLFEEILGGSGGGGSGGSSSGGSLLNPVLLPPKVKAYLSQGERFIKWDDETTVASPVILRVDPKGYYLYWTYQSKEMEFLDITSIRDTRFGKFAKMPKSQKLRDVFNMDFPDNSFLLKTLTVVSGPDMVDLTFHNFVSYKENVGKAWAEDVLALVKHPLTANASRSTFLDKILVKLKMQLNSEGKIPVKNFFQMFPADRKRVEAALSACHLPKGKNDAINPEDFPEPVYKSFLMSLCPRPEIDEIFTSYHAKAKPYMTKEHLTKFINQKQRDSRLNSLLFPPARPDQVQGLIDKYEPSGINAQRGQLSPEGMVWFLCGPENSVLAQDKLLLHHDMTQPLNHYFINSSHNTYLTAGQFSGLSSAEMYRQVLLSGCRCVELDCWKGKPPDEEPIITHGFTMTTDIFFKEAIEAIAESAFKTSPYPIILSFENHVDSPRQQAKMAEYCRTIFGDMLLTEPLEKFPLKPGVPLPSPEDLRGKILIKNKKNQFSGPTSSSKDTGGEAEGSSPPSAPAVWAGEEGTELEEEEVEEEEEEESGNLDEEEIKKMQSDEGTAGLEVTAYEEMSSLVNYIQPTKFVSFEFSAQKNRSYVISSFTELKAYDLLSKASVQFVDYNKRQMSRIYPKGTRMDSSNYMPQMFWNAGCQMVALNFQTMDLPMQQNMAVFEFNGQSGYLLKHEFMRRPDKQFNPFSVDRIDVVVATTLSITVISGQFLSERSVRTYVEVELFGLPGDPKRRYRTKLSPSTNSINPVWKEEPFVFEKILMPELASLRVAVMEEGNKFLGHRIIPINALNSGYHHLCLHSESNMPLTMPALFIFLEMKDYIPGAWADLTVALANPIKFFSAHDTKSVKLKEAMGGLPEKPFPLASPVASQVNGALAPTSNGSPAARAGAREEAMKEAAEPRTASLEELRELKGVVKLQRRHEKELRELERRGARRWEELLQRGAAQLAELGPPGVGGVGACKLGPGKGSRKKRSLPREESAGAAPGEGPEGVDGRVRELKDRLELELLRQGEEQYECVLKRKEQHVAEQISKMMELAREKQAAELKALKETSENDTKEMKKKLETKRLERIQGMTKVTTDKMAQERLKREINNSHIQEVVQVIKQMTENLERHQEKLEEKQAACLEQIREMEKQFQKEALAEYEARMKGLEAEVKESVRACLRTCFPSEAKDKPERACECPPELCEQDPLIAKADAQESRL

SEQ ID NO: 47 - protein, 1260 aa, Homo sapiens
MVTGYRLFEEILGGSGGGGSGGSSSGGAGAQPGVHALQLEPPTVVETLRRGSKFIKWDEETSSRNLVTLRVDPNGFFLYWTGPNMEVDTLDISSIRDTRTGRYARLPKDPKIREVLGFGGPDARLEEKLMTVVSGPDPVNTVFLNFMAVQDDTAKVWSEELFKLAMNILAQNASRNTFLRKAYTKLKLQVNQDGRIPVKNILKMFSADKKRVETALESCGLKFNRSESIRPDEFSLEIFERFLNKLCLRPDIDKILLEIGAKGKPYLTLEQLMDFINQKQRDPRLNEVLYPPLRPSQARLLIEKYEPNQQFLERDQMSMEGFSRYLGGEENGILPLEALDLSTDMTQPLSAYFINSSHNTYLTAGQLAGTSSVEMYRQALLWGCRCVELDVWKGRPPEEEPFITHGFTMTTEVPLRDVLEAIAETAFKTSPYPVILSFENHVDSAKQQAKMAEYCRSIFGDALLIEPLDKYPLAPGVPLPSPQDLMGRILVKNKKRHRPSAGGPDSAGRKRPLEQSNSALSESSAATEPSSPQLGSPSSDSCPGLSNGEEVGLEKPSLEPQKSLGDEGLNRGPYVLGPADREDEEEDEEEEEQTDPKKPTTDEGTASSEVNATEEMSTLVNYIEPVKFKSFEAARKRNKCFEMSSFVETKAMEQLTKSPMEFVEYNKQQLSRIYPKGTRVDSSNYMPQLFWNVGCQLVALNFQTLDVAMQLNAGVFEYNGRSGYLLKPEFMRRPDKSFDPFTEVIVDGIVANALRVKVISGQFLSDRKVGIYVEVDMFGLPVDTRRKYRTRTSQGNSFNPVWDEEPFDFPKVVLPTLASLRIAAFEEGGKFVGHRILPVSAIRSGYHYVCLRNEANQPLCLPALLIYTEASDYIPDDHQDYAEALINPIKHVSLMDQRARQLAALIGESEAQAGQETCQDTQSQQLGSQPSSNPTPSPLDASPRRPPGPTTSPASTSLSSPGQRDDLIASILSEVAPTPLDELRGHKALVKLRSRQERDLRELRKKHQRKAVTLTRRLLDGLAQAQAEGRCRLRPGALGGAADVEDTKEGEDEAKRYQEFQNRQVQSLLELREAQVDAEAQRRLEHLRQALQRLREVVLDANTTQFKRLKEMNEREKKELQKILDRKRHNSISEAKMRDKHKKEAELTEINRRHITESVNSIRRLEEAQKQRHDRLVAGQQQVLQQLAEEEPKLLAQLAQECQEQRARLPQEIRRSLLGEMPEGLGDGPLVACASNGHAPGSSGHLSGADSESQEENTQL

SEQ ID NO: 48 - protein, 1220 aa, Homo sapiens
MVTGYRLFEEILGGSGGGGSGGSSSGGAKPYEFNWQKEVPSFLQEGAVFDRYEEESFVFEPNCLFKVDEFGFFLTWRSEGKEGQVLECSLINSIRSGAIPKDPKILAALEAVGKSENDLEGRIVCVCSGTDLVNISFTYMVAENPEVTKQWVEGLRSIIHNFRANNVSPMTCLKKHWMKLAFMTNTNGKIPVRSITRTFASGKTEKVIFQALKELGLPSGKNDEIEPTAFSYEKFYELTQKICPRTDIEDLFKKINGDKTDYLTVDQLVSFLNEHQRDPRLNEILFPFYDAKRAMQIIEMYEPDEDLKKKGLISSDGFCRYLMSDENAPVFLDRLELYQEMDHPLAHYFISSSHNTYLTGRQFGGKSSVEMYRQVLLAGCRCVELDCWDGKGEDQEPIITHGKAMCTDILFKDVIQAIKETAFVTSEYPVILSFENHCSKYQQYKMSKYCEDLFGDLLLKQALESHPLEPGRALPSPNDLKRKILIKNKRLKPEVEKKQLEALRSMMEAGESASPANILEDDNEEEIESADQEEEAHPEFKFGNELSADDLGHKEAVANSVKKGLVTVEDEQAWMASYKYVGATTNIHPYLSTMINYAQPVKFQGFHVAEERNIHYNMSSFNESVGLGYLKTHAIEFVNYNKRQMSRIYPKGGRVDSSNYMPQIFWNAGCQMVSLNYQTPDLAMQLNQGKFEYNGSCGYLLKPDFMRRPDRTFDPFSETPVDGVIAATCSVQVISGQFLSDKKIGTYVEVDMYGLPTDTIRKEFRTRMVMNNGLNPVYNEESFVFRKVILPDLAVLRIAVYDDNNKLIGQRILPLDGLQAGYRHISLRNEGNKPLSLPTIFCNIVLKTYVPDGFGDIVDALSDPKKFLSITEKRADQMRAMGIETSDIADVPSDTSKNDKKGKANTAKANVTPQSSSELRPTTTAALASGVEAKKGIELIPQVRIEDLKQMKAYLKHLKKQQKELNSLKKKHAKEHSTMQKLHCTQVDKIVAQYDKEKSTHEKILEKAMKKKGGSNCLEMKKETEIKIQTLTSDHKSKVKEIVAQHTKEWSEMINTHSAEEQEIRDLHLSQQCELLKKLLINAHEQQTQQLKLSHDRESKEMRAHQAKISMENSKAISQDKSIKNKAERERRVRELNSSNTKKFLEERKRLAMKQSKEMDQLKKVQLEHLEFLEKQNEQLLKSCHAVSQTQGEGDAADGEIGSRDGPQTSNSSMKLQNAN

SEQ ID NO: 49 - protein, 158 aa, Homo sapiens
VFTLEDFVGDWEQTAAYNLDQVLEQGGVSSLLQNLAVSVTPIQRIVRSGENALKIDIHVIIPYEGLSADQMAQIEEVFKVVYPVDDHHFKVILPYGTLVIDGVTPNMLNYFGRPYEGIAVFDGKKITVTGTLWNGNKIIDERLITPDGSMLFRVTINS

SEQ ID NO: 50 - protein, 12 aa, Homo sapiens
MVTGYRLFEEIL

SEQ ID NO: 51 - protein, 15 aa, Homo sapiens
GGSGGGGSGGSSSGG

SEQ ID NO: 52 - protein, 8 aa, Homo sapiens
DYKDDDDK

SEQ ID NO: 53 - protein, 14 aa, Homo sapiens
RTAKQNPLTEKSGV

SEQ ID NO: 54 - protein, 9 aa, Homo sapiens
QSMGLSAAQ

SEQ ID NO: 55 - protein, 367 aa, Homo sapiens
MVFTLEDFVGDWEQTAAYNLDQVLEQGGVSSLLQNLAVSVTPIQRIVRSGENALKIDIHVIIPYEGLSADQMAQIEEVFKVVYPVDDHHFKVILPYGTLVIDGVTPNMLNYFGRPYEGIAVFDGKKITVTGTLWNGNKIIDERLITPDGSMLFRVTINSGGSGGGGSGGSSSGGTAAIRKKLVIVGDGACGKTCLLIVFSKDQFPEVYVPTVFENYVADIEVDGKQVELALWDTAGQEDYDRLRPLSYPDTDVILMCFSIDSPDSLENIPEKWTPEVKHFCPNVPIILVGNKKDLRNDEHTRRELAKMKQEPVKPEEGRDMANRIGAFGYMECSAKTKDGVREVFEMATRAALQARRGKKKSGCLVL

SEQ ID NO: 56 - protein, 127 aa, Homo sapiens
MVTGYRLFEEILGGSGGGGSGGSSSGGESEPRSWSLLEQLGLAGADLAAPGVQQQLELERERLRREIRKELKLKEGAENLRRATTDLGRSLGPVELLLRGSSRRLDLLHQQLQELHAHVVLPDPAAT

SEQ ID NO: 57 - protein, 581 aa, Homo sapiens
MVFTLEDFVGDWEQTAAYNLDQVLEQGGVSSLLQNLAVSVTPIQRIVRSGENALKIDIHVIIPYEGLSADQMAQIEEVFKVVYPVDDHHFKVILPYGTLVIDGVTPNMLNYFGRPYEGIAVFDGKKITVTGTLWNGNKIIDERLITPDGSMLFRVTINSGGSGGGGSGGSSSGGTKYSSYREDVLKGGDVVRLFHAEQEKFLTCDEYEKKQHIFLRTTLRQSATSATSSKALWEIEVVHHDPCRGGAGQWNSLFRFKHLATGNYLAAELNPDYRDAQNEGKNVRDGVPPTSKKKRQAGEKIMYTLVSVPHGNDIASLFELDATTLQRADCLVPRNSYVRLRHLCTNTWVTSTSIPIDTDEERPVMLKIGTCQTKEDKEAFAIVSVPLSEVRDLDFANDANKVLATTVKKLENGTITQNERRFVTKLLEDLIFFVADVPNNGQEVLDVVITKPNRERQKLMREQNILAQVFGILKAPFKEKAGEGSMLRLEDLGDQRYAPYKYMLRLCYRVLRHSQQDYRKNQEYIAKNFCVMQSQIGYDILAEDTITALLHNNRKGGSGGGGSGGSSSGGVTGYRLFEEIL

SEQ ID NO: 58 - protein, 352 aa, Homo sapiens
MTLESIMACCLSEEAKEARRINDEIERQLRRDKRDARRELKLLLLGTGESGKSTFIKQMRIIHGSGYSDEDKRGFTKLVYQNIFTAMQAMIRAMDTLKIPYKYEHNKAHAQLVREVDVEKVSAFENPYVDAIKSLWNDPGIQECYDRRREYQLSDSTKYYLNDLDRVADPAYLPTQQDVLRVRVPTTGIIEYPFDLQSVIFRMVDVGGQRSERRKWIHCFENVTSIMFLVALSEYDQVLVESDNENRMEESKALFRTIITYPWFQNSSVILFLNKKDLLEEKIMYSHLVDYFPEYDGPQRDAQAAREFILKMFVDLNPDSDKIIYSHFTCATDTENIRFVFAAVKDTILQLN

SEQ ID NO: 59 - protein, 359 aa, Homo sapiens
MTLESIMACCLSEEAKEARRINDEIERQLRRDKRDARRELKLLLLGTGESGKSTFIKQMRIIHGSGYSDEDKRGFTKLVYQNIFTAMQAMIRAMDTLKIPYKYEHNKAHAQLVREVDVEKVSAFENPYVDAIKSLWNDPGIQECYDRRREYQLSDSTKYYLNDLDRVADPAYLPTQQDVLRVRVPTTGIIEYPFDLQSVIFRMVDVGGQRSERRKWIHCFENVTSIMFLVALSEYDQVLVESDNENRMEESKALFRTIITYPWFQNSSVILFLNKKDLLEEKIMYSHLVDYFPEYDGPQRDAQAAREFILKMFVDLNPDSDKIIYSHFTCATDTENIRFVFAAVKDTILQLNLRQYELL

SEQ ID NO: 60 - protein, 359 aa, Homo sapiens
MTLESIMACCLSEEAKEARRINDEIERQLRRDKRDARRELKLLLLGTGESGKSTFIKQMRIIHGSGYSDEDKRGFTKLVYQNIFTAMQAMIRAMDTLKIPYKYEHNKAHAQLVREVDVEKVSAFENPYVDAIKSLWNDPGIQECYDRRREYQLSDSTKYYLNDLDRVADPAYLPTQQDVLRVRVPTTGIIEYPFDLQSVIFRMVDVGGQRSERRKWIHCFENVTSIMFLVALSEYDQVLVESDNENRMEESKALFRTIITYPWFQNSSVILFLNKKDLLEEKIMYSHLVDYFPEYDGPQRDAQAAREFILKMFVDLNPDSDKIIYSHFTCATDTENIRFVFAAVKDTILQLNLKQYELL

SEQ ID NO: 61 - protein, 359 aa, Homo sapiens
MTLESIMACCLSEEAKEARRINDEIERQLRRDKRDARRELKLLLLGTGESGKSTFIKQMRIIHGSGYSDEDKRGFTKLVYQNIFTAMQAMIRAMDTLKIPYKYEHNKAHAQLVREVDVEKVSAFENPYVDAIKSLWNDPGIQECYDRRREYQLSDSTKYYLNDLDRVADPAYLPTQQDVLRVRVPTTGIIEYPFDLQSVIFRMVDVGGQRSERRKWIHCFENVTSIMFLVALSEYDQVLVESDNENRMEESKALFRTIITYPWFQNSSVILFLNKKDLLEEKIMYSHLVDYFPEYDGPQRDAQAAREFILKMFVDLNPDSDKIIYSHFTCATDTENIRFVFAAVKDTILQLNLKDCGLF

SEQ ID NO: 62 - protein, 359 aa, Homo sapiens
MTLESIMACCLSEEAKEARRINDEIERQLRRDKRDARRELKLLLLGTGESGKSTFIKQMRIIHGSGYSDEDKRGFTKLVYQNIFTAMQAMIRAMDTLKIPYKYEHNKAHAQLVREVDVEKVSAFENPYVDAIKSLWNDPGIQECYDRRREYQLSDSTKYYLNDLDRVADPAYLPTQQDVLRVRVPTTGIIEYPFDLQSVIFRMVDVGGQRSERRKWIHCFENVTSIMFLVALSEYDQVLVESDNENRMEESKALFRTIITYPWFQNSSVILFLNKKDLLEEKIMYSHLVDYFPEYDGPQRDAQAAREFILKMFVDLNPDSDKIIYSHFTCATDTENIRFVFAAVKDTILQLNLKECGLY

SEQ ID NO: 63 - protein, 359 aa, Homo sapiens
MTLESIMACCLSEEAKEARRINDEIERQLRRDKRDARRELKLLLLGTGESGKSTFIKQMRIIHGSGYSDEDKRGFTKLVYQNIFTAMQAMIRAMDTLKIPYKYEHNKAHAQLVREVDVEKVSAFENPYVDAIKSLWNDPGIQECYDRRREYQLSDSTKYYLNDLDRVADPAYLPTQQDVLRVRVPTTGIIEYPFDLQSVIFRMVDVGGQRSERRKWIHCFENVTSIMFLVALSEYDQVLVESDNENRMEESKALFRTIITYPWFQNSSVILFLNKKDLLEEKIMYSHLVDYFPEYDGPQRDAQAAREFILKMFVDLNPDSDKIIYSHFTCATDTENIRFVFAAVKDTILQLNLRGCGLY

SEQ ID NO: 64 - protein, 359 aa, Homo sapiens
MTLESIMACCLSEEAKEARRINDEIERQLRRDKRDARRELKLLLLGTGESGKSTFIKQMRIIHGSGYSDEDKRGFTKLVYQNIFTAMQAMIRAMDTLKIPYKYEHNKAHAQLVREVDVEKVSAFENPYVDAIKSLWNDPGIQECYDRRREYQLSDSTKYYLNDLDRVADPAYLPTQQDVLRVRVPTTGIIEYPFDLQSVIFRMVDVGGQRSERRKWIHCFENVTSIMFLVALSEYDQVLVESDNENRMEESKALFRTIITYPWFQNSSVILFLNKKDLLEEKIMYSHLVDYFPEYDGPQRDAQAAREFILKMFVDLNPDSDKIIYSHFTCATDTENIRFVFAAVKDTILQLNLKYIGLC

SEQ ID NO: 65 - protein, 359 aa, Homo sapiens
MTLESIMACCLSEEAKEARRINDEIERQLRRDKRDARRELKLLLLGTGESGKSTFIKQMRIIHGSGYSDEDKRGFTKLVYQNIFTAMQAMIRAMDTLKIPYKYEHNKAHAQLVREVDVEKVSAFENPYVDAIKSLWNDPGIQECYDRRREYQLSDSTKYYLNDLDRVADPAYLPTQQDVLRVRVPTTGIIEYPFDLQSVIFRMVDVGGQRSERRKWIHCFENVTSIMFLVALSEYDQVLVESDNENRMEESKALFRTIITYPWFQNSSVILFLNKKDLLEEKIMYSHLVDYFPEYDGPQRDAQAAREFILKMFVDLNPDSDKIIYSHFTCATDTENIRFVFAAVKDTILQLNLKEYNLV

SEQ ID NO: 66 - protein, 359 aa, Homo sapiens
MTLESIMACCLSEEAKEARRINDEIERQLRRDKRDARRELKLLLLGTGESGKSTFIKQMRIIHGSGYSDEDKRGFTKLVYQNIFTAMQAMIRAMDTLKIPYKYEHNKAHAQLVREVDVEKVSAFENPYVDAIKSLWNDPGIQECYDRRREYQLSDSTKYYLNDLDRVADPAYLPTQQDVLRVRVPTTGIIEYPFDLQSVIFRMVDVGGQRSERRKWIHCFENVTSIMFLVALSEYDQVLVESDNENRMEESKALFRTIITYPWFQNSSVILFLNKKDLLEEKIMYSHLVDYFPEYDGPQRDAQAAREFILKMFVDLNPDSDKIIYSHFTCATDTENIRFVFAAVKDTILQLNLREFNLV

SEQ ID NO: 67 - protein, 359 aa, Homo sapiens
MTLESIMACCLSEEAKEARRINDEIERQLRRDKRDARRELKLLLLGTGESGKSTFIKQMRIIHGSGYSDEDKRGFTKLVYQNIFTAMQAMIRAMDTLKIPYKYEHNKAHAQLVREVDVEKVSAFENPYVDAIKSLWNDPGIQECYDRRREYQLSDSTKYYLNDLDRVADPAYLPTQQDVLRVRVPTTGIIEYPFDLQSVIFRMVDVGGQRSERRKWIHCFENVTSIMFLVALSEYDQVLVESDNENRMEESKALFRTIITYPWFQNSSVILFLNKKDLLEEKIMYSHLVDYFPEYDGPQRDAQAAREFILKMFVDLNPDSDKIIYSHFTCATDTENIRFVFAAVKDTILQLNLDEINLL

SEQ ID NO: 68 - protein, 359 aa, Homo sapiens
MTLESIMACCLSEEAKEARRINDEIERQLRRDKRDARRELKLLLLGTGESGKSTFIKQMRIIHGSGYSDEDKRGFTKLVYQNIFTAMQAMIRAMDTLKIPYKYEHNKAHAQLVREVDVEKVSAFENPYVDAIKSLWNDPGIQECYDRRREYQLSDSTKYYLNDLDRVADPAYLPTQQDVLRVRVPTTGIIEYPFDLQSVIFRMVDVGGQRSERRKWIHCFENVTSIMFLVALSEYDQVLVESDNENRMEESKALFRTIITYPWFQNSSVILFLNKKDLLEEKIMYSHLVDYFPEYDGPQRDAQAAREFILKMFVDLNPDSDKIIYSHFTCATDTENIRFVFAAVKDTILQLNLKDIMLQ

SEQ ID NO: 69 - protein, 359 aa, Homo sapiens
MTLESIMACCLSEEAKEARRINDEIERQLRRDKRDARRELKLLLLGTGESGKSTFIKQMRIIHGSGYSDEDKRGFTKLVYQNIFTAMQAMIRAMDTLKIPYKYEHNKAHAQLVREVDVEKVSAFENPYVDAIKSLWNDPGIQECYDRRREYQLSDSTKYYLNDLDRVADPAYLPTQQDVLRVRVPTTGIIEYPFDLQSVIFRMVDVGGQRSERRKWIHCFENVTSIMFLVALSEYDQVLVESDNENRMEESKALFRTIITYPWFQNSSVILFLNKKDLLEEKIMYSHLVDYFPEYDGPQRDAQAAREFILKMFVDLNPDSDKIIYSHFTCATDTENIRFVFAAVKDTILQLNLKQLMLQ

SEQ ID NO: 70 - protein, 374 aa, Homo sapiens
MGCLGNSKTEDQRNEEKAQREANKKIEKQLQKDKQVYRATHRLLLLGAGESGKSTIVKQMRILHVNGFNGDSEKATKVQDIKNNLKEAIETIVAAMSNLVPPVELANPENQFRVDYILSVMNVPDFDFPPEFYEHAKALWEDEGVRACYERSNEYQLIDCAQYFLDKIDVIKQADYVPSDQDLLRCRVLTSGIFETKFQVDKVNFHMFDVGGQRDERRKWIQCFNDVTAIIFVVASSSYNMVIREDNQTNRLQEALNLFKSIWNNRWLRTISVILFLNKQDLLAEKVLAGKSKIEDYFPEFARYTTPEDATPEPGEDPRVTRAKYFIRDEFLRISTASGDGRHYCYPHFTCAVDTENIRRVFNDCRDIIQRMHL

SEQ ID NO: 71 - protein, 380 aa, Homo sapiens
MGCLGNSKTEDQRNEEKAQREANKKIEKQLQKDKQVYRATHRLLLLGAGESGKSTIVKQMRILHVNGFNGDSEKATKVQDIKNNLKEAIETIVAAMSNLVPPVELANPENQFRVDYILSVMNVPDFDFPPEFYEHAKALWEDEGVRACYERSNEYQLIDCAQYFLDKIDVIKQADYVPSDQDLLRCRVLTSGIFETKFQVDKVNFHMFDVGGQRDERRKWIQCFNDVTAIIFVVASSSYNMVIREDNQTNRLQEALNLFKSIWNNRWLRTISVILFLNKQDLLAEKVLAGKSKIEDYFPEFARYTTPEDATPEPGEDPRVTRAKYFIRDEFLRISTASGDGRHYCYPHFTCAVDTENIRRVFNDCRDIIQRMHLRQYELL

SEQ ID NO: 72 - protein, 380 aa, Homo sapiens
MGCLGNSKTEDQRNEEKAQREANKKIEKQLQKDKQVYRATHRLLLLGAGESGKSTIVKQMRILHVNGFNGDSEKATKVQDIKNNLKEAIETIVAAMSNLVPPVELANPENQFRVDYILSVMNVPDFDFPPEFYEHAKALWEDEGVRACYERSNEYQLIDCAQYFLDKIDVIKQADYVPSDQDLLRCRVLTSGIFETKFQVDKVNFHMFDVGGQRDERRKWIQCFNDVTAIIFVVASSSYNMVIREDNQTNRLQEALNLFKSIWNNRWLRTISVILFLNKQDLLAEKVLAGKSKIEDYFPEFARYTTPEDATPEPGEDPRVTRAKYFIRDEFLRISTASGDGRHYCYPHFTCAVDTENIRRVFNDCRDIIQRMHLKDCGLF

SEQ ID NO: 73 - protein, 380 aa, Homo sapiens
MGCLGNSKTEDQRNEEKAQREANKKIEKQLQKDKQVYRATHRLLLLGAGESGKSTIVKQMRILHVNGFNGDSEKATKVQDIKNNLKEAIETIVAAMSNLVPPVELANPENQFRVDYILSVMNVPDFDFPPEFYEHAKALWEDEGVRACYERSNEYQLIDCAQYFLDKIDVIKQADYVPSDQDLLRCRVLTSGIFETKFQVDKVNFHMFDVGGQRDERRKWIQCFNDVTAIIFVVASSSYNMVIREDNQTNRLQEALNLFKSIWNNRWLRTISVILFLNKQDLLAEKVLAGKSKIEDYFPEFARYTTPEDATPEPGEDPRVTRAKYFIRDEFLRISTASGDGRHYCYPHFTCAVDTENIRRVFNDCRDIIQRMHLKECGLY

SEQ ID NO: 74 - protein, 380 aa, Homo sapiens
MGCLGNSKTEDQRNEEKAQREANKKIEKQLQKDKQVYRATHRLLLLGAGESGKSTIVKQMRILHVNGFNGDSEKATKVQDIKNNLKEAIETIVAAMSNLVPPVELANPENQFRVDYILSVMNVPDFDFPPEFYEHAKALWEDEGVRACYERSNEYQLIDCAQYFLDKIDVIKQADYVPSDQDLLRCRVLTSGIFETKFQVDKVNFHMFDVGGQRDERRKWIQCFNDVTAIIFVVASSSYNMVIREDNQTNRLQEALNLFKSIWNNRWLRTISVILFLNKQDLLAEKVLAGKSKIEDYFPEFARYTTPEDATPEPGEDPRVTRAKYFIRDEFLRISTASGDGRHYCYPHFTCAVDTENIRRVFNDCRDIIQRMHLRGCGLY

SEQ ID NO: 75 - protein, 380 aa, Homo sapiens
MGCLGNSKTEDQRNEEKAQREANKKIEKQLQKDKQVYRATHRLLLLGAGESGKSTIVKQMRILHVNGFNGDSEKATKVQDIKNNLKEAIETIVAAMSNLVPPVELANPENQFRVDYILSVMNVPDFDFPPEFYEHAKALWEDEGVRACYERSNEYQLIDCAQYFLDKIDVIKQADYVPSDQDLLRCRVLTSGIFETKFQVDKVNFHMFDVGGQRDERRKWIQCFNDVTAIIFVVASSSYNMVIREDNQTNRLQEALNLFKSIWNNRWLRTISVILFLNKQDLLAEKVLAGKSKIEDYFPEFARYTTPEDATPEPGEDPRVTRAKYFIRDEFLRISTASGDGRHYCYPHFTCAVDTENIRRVFNDCRDIIQRMHLKYIGLC

SEQ ID NO: 76 - protein, 380 aa, Homo sapiens
MGCLGNSKTEDQRNEEKAQREANKKIEKQLQKDKQVYRATHRLLLLGAGESGKSTIVKQMRILHVNGFNGDSEKATKVQDIKNNLKEAIETIVAAMSNLVPPVELANPENQFRVDYILSVMNVPDFDFPPEFYEHAKALWEDEGVRACYERSNEYQLIDCAQYFLDKIDVIKQADYVPSDQDLLRCRVLTSGIFETKFQVDKVNFHMFDVGGQRDERRKWIQCFNDVTAIIFVVASSSYNMVIREDNQTNRLQEALNLFKSIWNNRWLRTISVILFLNKQDLLAEKVLAGKSKIEDYFPEFARYTTPEDATPEPGEDPRVTRAKYFIRDEFLRISTASGDGRHYCYPHFTCAVDTENIRRVFNDCRDIIQRMHLKEYNLV

SEQ ID NO: 77 - protein, 380 aa, Homo sapiens
MGCLGNSKTEDQRNEEKAQREANKKIEKQLQKDKQVYRATHRLLLLGAGESGKSTIVKQMRILHVNGFNGDSEKATKVQDIKNNLKEAIETIVAAMSNLVPPVELANPENQFRVDYILSVMNVPDFDFPPEFYEHAKALWEDEGVRACYERSNEYQLIDCAQYFLDKIDVIKQADYVPSDQDLLRCRVLTSGIFETKFQVDKVNFHMFDVGGQRDERRKWIQCFNDVTAIIFVVASSSYNMVIREDNQTNRLQEALNLFKSIWNNRWLRTISVILFLNKQDLLAEKVLAGKSKIEDYFPEFARYTTPEDATPEPGEDPRVTRAKYFIRDEFLRISTASGDGRHYCYPHFTCAVDTENIRRVFNDCRDIIQRMHLREFNLV

SEQ ID NO: 78 - protein, 380 aa, Homo sapiens
MGCLGNSKTEDQRNEEKAQREANKKIEKQLQKDKQVYRATHRLLLLGAGESGKSTIVKQMRILHVNGFNGDSEKATKVQDIKNNLKEAIETIVAAMSNLVPPVELANPENQFRVDYILSVMNVPDFDFPPEFYEHAKALWEDEGVRACYERSNEYQLIDCAQYFLDKIDVIKQADYVPSDQDLLRCRVLTSGIFETKFQVDKVNFHMFDVGGQRDERRKWIQCFNDVTAIIFVVASSSYNMVIREDNQTNRLQEALNLFKSIWNNRWLRTISVILFLNKQDLLAEKVLAGKSKIEDYFPEFARYTTPEDATPEPGEDPRVTRAKYFIRDEFLRISTASGDGRHYCYPHFTCAVDTENIRRVFNDCRDIIQRMHLDEINLL

SEQ ID NO: 79 - protein, 380 aa, Homo sapiens
MGCLGNSKTEDQRNEEKAQREANKKIEKQLQKDKQVYRATHRLLLLGAGESGKSTIVKQMRILHVNGFNGDSEKATKVQDIKNNLKEAIETIVAAMSNLVPPVELANPENQFRVDYILSVMNVPDFDFPPEFYEHAKALWEDEGVRACYERSNEYQLIDCAQYFLDKIDVIKQADYVPSDQDLLRCRVLTSGIFETKFQVDKVNFHMFDVGGQRDERRKWIQCFNDVTAIIFVVASSSYNMVIREDNQTNRLQEALNLFKSIWNNRWLRTISVILFLNKQDLLAEKVLAGKSKIEDYFPEFARYTTPEDATPEPGEDPRVTRAKYFIRDEFLRISTASGDGRHYCYPHFTCAVDTENIRRVFNDCRDIIQRMHLKDIMLQ

SEQ ID NO: 80 - protein, 380 aa, Homo sapiens
MGCLGNSKTEDQRNEEKAQREANKKIEKQLQKDKQVYRATHRLLLLGAGESGKSTIVKQMRILHVNGFNGDSEKATKVQDIKNNLKEAIETIVAAMSNLVPPVELANPENQFRVDYILSVMNVPDFDFPPEFYEHAKALWEDEGVRACYERSNEYQLIDCAQYFLDKIDVIKQADYVPSDQDLLRCRVLTSGIFETKFQVDKVNFHMFDVGGQRDERRKWIQCFNDVTAIIFVVASSSYNMVIREDNQTNRLQEALNLFKSIWNNRWLRTISVILFLNKQDLLAEKVLAGKSKIEDYFPEFARYTTPEDATPEPGEDPRVTRAKYFIRDEFLRISTASGDGRHYCYPHFTCAVDTENIRRVFNDCRDIIQRMHLKQLMLQ

SEQ ID NO: 81 - protein, 6 aa, Homo sapiens
RQYELL

SEQ ID NO: 82 - protein, 6 aa, Homo sapiens
KQYELL

SEQ ID NO: 83 - protein, 6 aa, Homo sapiens
KDCGLF

SEQ ID NO: 84 - protein, 6 aa, Homo sapiens
KECGLY

SEQ ID NO: 85 - protein, 6 aa, Homo sapiens
RGCGLY

SEQ ID NO: 86 - protein, 6 aa, Homo sapiens
KYIGLC

SEQ ID NO: 87 - protein, 6 aa, Homo sapiens
REFNLV

SEQ ID NO: 88 - protein, 6 aa, Homo sapiens
DEINLL

SEQ ID NO: 89 - protein, 6 aa, Homo sapiens
KDIMLQ

SEQ ID NO: 90 - protein, 6 aa, Homo sapiens
KQLMLQ

SEQ ID NO: 91 - protein, 6 aa, Homo sapiens
KEYNLV

SEQ ID NO: 92 - protein, 6 aa, Homo sapiens
KDIMLQ

SEQ ID NO: 93 - protein, 651 aa, Homo sapiens
MVPSAGQLALFALGIVLAACQALENSTSPLSADPPVAAAVVSRSGIIPVEEENPDFWNREAAEALGAAKKLQPAQTAAKNLIIFLGDGMGVSTVTAARILKGQKKDKLGPEIPLAMDRFPYVALSKTYNVDKHVPDSGATATAYLCGVKGNFQTIGLSAAARFNQCNTTRGNEVISVMNRAKKAGKSVGVVTTTRVQHASPAGTYAHTVNRNWYSDADVPASARQEGCQDIATQLISNMDIDVILGGGRKYMFRMGTPDPEYPDDYSQGGTRLDGKNLVQEWLAKRQGARYVWNRTELMQASLDPSVTHLMGLFEPGDMKYEIHRDSTLDPSLMEMTEAALRLLSRNPRGFFLFVEGGRIDHGHHESRAYRALTETIMFDDAIERAGQLTSEEDTLSLVTADHSHVFSFGGYPLRGSSIFGLAPGKARDRKAYTVLLYGNGPGYVLKDGARPDVTESESGSPEYRQQSAVPLDEETHAGEDVAVFARGPQAHLVHGVQEQTFIAHVMAFAACLEPYTACDLAPPAGTTDAAHPGYHDCPDSHTQFCFHGTCRFLVQEDKPACVCHSGYVGARCEHADLLAVVAASQKKQAITALVVVSIVALAVLIITCVLIHCCQVRKHCEWCRALICRHEKPSALLKGRTACCHSETVV

SEQ ID NO: 94 - protein, 39 aa, Homo sapiens
MVPSAGQLALFALGIVLAACQALENSTSPLSADPPVAAA

SEQ ID NO: 95 - protein, 489 aa, Homo sapiens
GIIPVEEENPDFWNREAAEALGAAKKLQPAQTAAKNLIIFLGDGMGVSTVTAARILKGQKKDKLGPEIPLAMDRFPYVALSKTYNVDKHVPDSGATATAYLCGVKGNFQTIGLSAAARFNQCNTTRGNEVISVMNRAKKAGKSVGVVTTTRVQHASPAGTYAHTVNRNWYSDADVPASARQEGCQDIATQLISNMDIDVILGGGRKYMFRMGTPDPEYPDDYSQGGTRLDGKNLVQEWLAKRQGARYVWNRTELMQASLDPSVTHLMGLFEPGDMKYEIHRDSTLDPSLMEMTEAALRLLSRNPRGFFLFVEGGRIDHGHHESRAYRALTETIMFDDAIERAGQLTSEEDTLSLVTADHSHVFSFGGYPLRGSSIFGLAPGKARDRKAYTVLLYGNGPGYVLKDGARPDVTESESGSPEYRQQSAVPLDEETHAGEDVAVFARGPQAHLVHGVQEQTFIAHVMAFAACLEPYTACDLAPPAGTTDAAHP

SEQ ID NO: 96 - protein, 48 aa, Homo sapiens
GYHDCPDSHTQFCFHGTCRFLVQEDKPACVCHSGYVGARCEHADLLAV

SEQ ID NO: 97 - RNA, 25 nt, Homo sapiens
  source 1..25: mol_type = unassigned RNA
ggagagagnggcaagagnacgnnna

SEQ ID NO: 98 - RNA, 25 nt, Homo sapiens
  source 1..25: mol_type = unassigned RNA
cccnnngacnnacaaagngncannn

SEQ ID NO: 99 - RNA, 25 nt, Homo sapiens
  source 1..25: mol_type = unassigned RNA
ccggcancancgagnacccnnncga

SEQ ID NO: 100 - RNA, 25 nt, Homo sapiens
  source 1..25: mol_type = unassigned RNA
gcancagnacgncagngccancaag

SEQ ID NO: 101 - RNA, 25 nt, Homo sapiens
  source 1..25: mol_type = unassigned RNA
ccancgncaacaacaagcncnncnn

SEQ ID NO: 102 - RNA, 25 nt, Homo sapiens
  source 1..25: mol_type = unassigned RNA
cagaagcccnnanaccaccacnnca

SEQ ID NO: 103 - RNA, 25 nt, Homo sapiens
  source 1..25: mol_type = unassigned RNA
gcagcccaaggaanggnggaaacaa

SEQ ID NO: 104 - RNA, 25 nt, Homo sapiens
  source 1..25: mol_type = unassigned RNA
cagaancgngnngacagcaaagaaa

SEQ ID NO: 105 - RNA, 21 nt, Homo sapiens
  source 1..21: mol_type = unassigned RNA
accgaatggaggaaagcaagg

SEQ ID NO: 106 - RNA, 25 nt, Homo sapiens
  source 1..25: mol_type = unassigned RNA
catctctctggggtccatcatattc

SEQ ID NO: 107 - RNA, 20 nt, Homo sapiens
  source 1..20: mol_type = unassigned RNA
cagcgaatacgaccaagtcc

SEQ ID NO: 108 - RNA, 20 nt, Homo sapiens
  source 1..20: mol_type = unassigned RNA
accaggggtaggtgatgatg

SEQ ID NO: 109 - RNA, 19 nt, Homo sapiens
  source 1..19: mol_type = unassigned RNA
gagggattctggcatcagg

SEQ ID NO: 110 - RNA, 19 nt, Homo sapiens
  source 1..19: mol_type = unassigned RNA
cgatccggtccaagttgtc

SEQ ID NO: 111 - RNA, 24 nt, Homo sapiens
  source 1..24: mol_type = unassigned RNA
cctggataacttggataaacttgg

SEQ ID NO: 112 - RNA, 19 nt, Homo sapiens
  source 1..19: mol_type = unassigned RNA
ttcatggatgcctttggtg

SEQ ID NO: 113 - RNA, 22 nt, Homo sapiens
  source 1..22: mol_type = unassigned RNA
gccaaggtcatccatgacaact

SEQ ID NO: 114 - RNA, 20 nt, Homo sapiens
  source 1..20: mol_type = unassigned RNA
gaggggccatccacagtctt